European Patent Application EP 4 549 563 A1, published May 7, 2025. Title: 중성 pH에서 활성을 나타내는 히알루로니다제 Hyal1 변이체. Applicant: Odysgen, Inc. Application KR. The sequence listing filed with the application follows.

SEQUENCE LISTING (50 sequences)

SEQ ID NO: 1 - protein, 435 aa, synthetic construct
MAAHLLPICALFLTLLDMAQGFRGPLLPNRPFTTVWNANTQWCLERHGVDVDVSVFDVVANPGQTFRGPDMTIFYSSQLGTYPYYTPTGEPVFGGLPQNASLIAHLARTFQDILAAIPAPDFSGLAVIDWEAWRPRWAFNWDTKDIYRQRSRALVQAQHPDWPAPQVEAVAQDQFQGAARAWMAGTLQLGRALRPRGLWGFYGFPDCYNYDFLSPNYTGQCPSGIRAQNDQLGWLWGQSRALYPSIYMPAVLEGTGKSQMYVQHRVAEAFRVAVAAGDPNLPVLPYVQIFYDTTNHFLPLDELEHSLGESAAQGAAGVVLWVSWENTRTKESCQAIKEYMDTTLGPFILNVTSGALLCSQALCSGHGRCVRRTSHPKALLLLNPASFSIQLTPGGGPLSLRGALSLEDQAQMAVEFKCRCYPGWQAPWCERKSMW

SEQ ID NO: 2 - protein, 435 aa, synthetic construct
MAAHLLPICALFLTLLDMAQGFRGPLLPNRPFTTVWNANTQWCLERHGVDVDVSVFDVVANPGQTFRGPDMTIFYSSQLGTYPYYTPTGEPVFGGLPQNASLIAHLARTFQDILAAIPAPDFSGLAVIDWEEWRPRWAFNWDTKDIYRQRSRALVQAQHPDWPAPQVEAVAQDQFQGAARAWMAGTLQLGRALRPRGLWGFYGFPDCYNYDFLSPNYTGQCPSGIRAQNDQLGWLWGQSRALYPSIYMPAVLEGTGKSQMYVQHRVAEAFRVAVAAGDPNLPVLPYVQIFYDTTNHFLPLDELEHSLGESAAQGAAGVVLWVSWENTRTKESCQAIKEYMDTTLGPFILNVTSGALLCSQALCSGHGRCVRRTSHPKALLLLNPASFSIQLTPGGGPLSLRGALSLEDQAQMAVEFKCRCYPGWQAPWCERKSMW

SEQ ID NO: 3 - protein, 435 aa, synthetic construct
MAAHLLPICALFLTLLDMAQGFRGPLLPNRPFTTVWNANTQWCLERHGVDVDVSVFDVVANPGQTFRGPDMTIFYSSQLGTYPYYTPTGEPVFGGLPQNASLIAHLARTFQDILAAIPAPDFSGLAVIDWENWRPRWAFNWDTKDIYRQRSRALVQAQHPDWPAPQVEAVAQDQFQGAARAWMAGTLQLGRALRPRGLWGFYGFPDCYNYDFLSPNYTGQCPSGIRAQNDQLGWLWGQSRALYPSIYMPAVLEGTGKSQMYVQHRVAEAFRVAVAAGDPNLPVLPYVQIFYDTTNHFLPLDELEHSLGESAAQGAAGVVLWVSWENTRTKESCQAIKEYMDTTLGPFILNVTSGALLCSQALCSGHGRCVRRTSHPKALLLLNPASFSIQLTPGGGPLSLRGALSLEDQAQMAVEFKCRCYPGWQAPWCERKSMW

SEQ ID NO: 4 - protein, 435 aa, synthetic construct
MAAHLLPICALFLTLLDMAQGFRGPLLPNRPFTTVWNANTQWCLERHGVDVDVSVFDVVANPGQTFRGPDMTIFYSSQLGTYPYYTPTGEPVFGGLPQNASLIAHLARTFQDILAAIPAPDFSGLAVIDWEDWRPRWAFNWDTKDIYRQRSRALVQAQHPDWPAPQVEAVAQDQFQGAARAWMAGTLQLGRALRPRGLWGFYGFPDCYNYDFLSPNYTGQCPSGIRAQNDQLGWLWGQSRALYPSIYMPAVLEGTGKSQMYVQHRVAEAFRVAVAAGDPNLPVLPYVQIFYDTTNHFLPLDELEHSLGESAAQGAAGVVLWVSWENTRTKESCQAIKEYMDTTLGPFILNVTSGALLCSQALCSGHGRCVRRTSHPKALLLLNPASFSIQLTPGGGPLSLRGALSLEDQAQMAVEFKCRCYPGWQAPWCERKSMW

SEQ ID NO: 5 - protein, 435 aa, synthetic construct
MAAHLLPICALFLTLLDMAQGFRGPLLPNRPFTTVWNANTQWCLERHGVDVDVSVFDVVANPGQTFRGPDMTIFYSSQLGTYPYYTPTGEPVFGGLPQNASLIAHLARTFQDILAAIPAPDFSGLAVIDWEYWRPRWAFNWDTKDIYRQRSRALVQAQHPDWPAPQVEAVAQDQFQGAARAWMAGTLQLGRALRPRGLWGFYGFPDCYNYDFLSPNYTGQCPSGIRAQNDQLGWLWGQSRALYPSIYMPAVLEGTGKSQMYVQHRVAEAFRVAVAAGDPNLPVLPYVQIFYDTTNHFLPLDELEHSLGESAAQGAAGVVLWVSWENTRTKESCQAIKEYMDTTLGPFILNVTSGALLCSQALCSGHGRCVRRTSHPKALLLLNPASFSIQLTPGGGPLSLRGALSLEDQAQMAVEFKCRCYPGWQAPWCERKSMW

SEQ ID NO: 6 - protein, 435 aa, synthetic construct
MAAHLLPICALFLTLLDMAQGFRGPLLPNRPFTTVWNANTQWCLERHGVDVDVSVFDVVANPGQTFRGPDMTIFYSSQLGTYPYYTPTGEPVFGGLPQNASLIAHLARTFQDILAAIPAPDFSGLAVIDWESWRPRWAFNWDTKDIYRQRSRALVQAQHPDWPAPQVEAVAQDQFQGAARAWMAGTLQLGRALRPRGLWGFYGFPDCYNYDFLSPNYTGQCPSGIRAQNDQLGWLWGQSRALYPSIYMPAVLEGTGKSQMYVQHRVAEAFRVAVAAGDPNLPVLPYVQIFYDTTNHFLPLDELEHSLGESAAQGAAGVVLWVSWENTRTKESCQAIKEYMDTTLGPFILNVTSGALLCSQALCSGHGRCVRRTSHPKALLLLNPASFSIQLTPGGGPLSLRGALSLEDQAQMAVEFKCRCYPGWQAPWCERKSMW

SEQ ID NO: 7 - protein, 435 aa, synthetic construct
MAAHLLPICALFLTLLDMAQGFRGPLLPNRPFTTVWNANTQWCLERHGVDVDVSVFDVVANPGQTFRGPDMTIFYSSQLGTYPYYTPTGEPVFGGLPQNASLIAHLARTFQDILAAIPAPDFSGLAVIDWEHWRPRWAFNWDTKDIYRQRSRALVQAQHPDWPAPQVEAVAQDQFQGAARAWMAGTLQLGRALRPRGLWGFYGFPDCYNYDFLSPNYTGQCPSGIRAQNDQLGWLWGQSRALYPSIYMPAVLEGTGKSQMYVQHRVAEAFRVAVAAGDPNLPVLPYVQIFYDTTNHFLPLDELEHSLGESAAQGAAGVVLWVSWENTRTKESCQAIKEYMDTTLGPFILNVTSGALLCSQALCSGHGRCVRRTSHPKALLLLNPASFSIQLTPGGGPLSLRGALSLEDQAQMAVEFKCRCYPGWQAPWCERKSMW

SEQ ID NO: 8 - protein, 435 aa, synthetic construct
MAAHLLPICALFLTLLDMAQGFRGPLLPNRPFTTVWNANTQWCLERHGVDVDVSVFDVVANPGQTFRGPDMTIFYSDQLGTYPYYTPTGEPVFGGLPQNASLIAHLARTFQDILAAIPAPDFSGLAVIDWEAWRPRWAFNWDTKDIYRQRSRALVQAQHPDWPAPQVEAVAQDQFQGAARAWMAGTLQLGRALRPRGLWGFYGFPDCYNYDFLSPNYTGQCPSGIRAQNDQLGWLWGQSRALYPSIYMPAVLEGTGKSQMYVQHRVAEAFRVAVAAGDPNLPVLPYVQIFYDTTNHFLPLDELEHSLGESAAQGAAGVVLWVSWENTRTKESCQAIKEYMDTTLGPFILNVTSGALLCSQALCSGHGRCVRRTSHPKALLLLNPASFSIQLTPGGGPLSLRGALSLEDQAQMAVEFKCRCYPGWQAPWCERKSMW

SEQ ID NO: 9 - protein, 435 aa, synthetic construct
MAAHLLPICALFLTLLDMAQGFRGPLLPNRPFTTVWNANTQWCLERHGVDVDVSVFDVVANPGQTFRGPDMTIFYSEQLGTYPYYTPTGEPVFGGLPQNASLIAHLARTFQDILAAIPAPDFSGLAVIDWEAWRPRWAFNWDTKDIYRQRSRALVQAQHPDWPAPQVEAVAQDQFQGAARAWMAGTLQLGRALRPRGLWGFYGFPDCYNYDFLSPNYTGQCPSGIRAQNDQLGWLWGQSRALYPSIYMPAVLEGTGKSQMYVQHRVAEAFRVAVAAGDPNLPVLPYVQIFYDTTNHFLPLDELEHSLGESAAQGAAGVVLWVSWENTRTKESCQAIKEYMDTTLGPFILNVTSGALLCSQALCSGHGRCVRRTSHPKALLLLNPASFSIQLTPGGGPLSLRGALSLEDQAQMAVEFKCRCYPGWQAPWCERKSMW

SEQ ID NO: 10 - protein, 435 aa, synthetic construct
MAAHLLPICALFLTLLDMAQGFRGPLLPNRPFTTVWNANTQWCLERHGVDVDVSVFDVVANPGQTFRGPDMTIFYSSQLGTYPYYDPTGEPVFGGLPQNASLIAHLARTFQDILAAIPAPDFSGLAVIDWEAWRPRWAFNWDTKDIYRQRSRALVQAQHPDWPAPQVEAVAQDQFQGAARAWMAGTLQLGRALRPRGLWGFYGFPDCYNYDFLSPNYTGQCPSGIRAQNDQLGWLWGQSRALYPSIYMPAVLEGTGKSQMYVQHRVAEAFRVAVAAGDPNLPVLPYVQIFYDTTNHFLPLDELEHSLGESAAQGAAGVVLWVSWENTRTKESCQAIKEYMDTTLGPFILNVTSGALLCSQALCSGHGRCVRRTSHPKALLLLNPASFSIQLTPGGGPLSLRGALSLEDQAQMAVEFKCRCYPGWQAPWCERKSMW

SEQ ID NO: 11 - protein, 435 aa, synthetic construct
MAAHLLPICALFLTLLDMAQGFRGPLLPNRPFTTVWNANTQWCLERHGVDVDVSVFDVVANPGQTFRGPDMTIFYSSQLGTYPYYEPTGEPVFGGLPQNASLIAHLARTFQDILAAIPAPDFSGLAVIDWEAWRPRWAFNWDTKDIYRQRSRALVQAQHPDWPAPQVEAVAQDQFQGAARAWMAGTLQLGRALRPRGLWGFYGFPDCYNYDFLSPNYTGQCPSGIRAQNDQLGWLWGQSRALYPSIYMPAVLEGTGKSQMYVQHRVAEAFRVAVAAGDPNLPVLPYVQIFYDTTNHFLPLDELEHSLGESAAQGAAGVVLWVSWENTRTKESCQAIKEYMDTTLGPFILNVTSGALLCSQALCSGHGRCVRRTSHPKALLLLNPASFSIQLTPGGGPLSLRGALSLEDQAQMAVEFKCRCYPGWQAPWCERKSMW

SEQ ID NO: 12 - protein, 435 aa, synthetic construct
MAAHLLPICALFLTLLDMAQGFRGPLLPNRPFTTVWNANTQWCLERHGVDVDVSVFDVVANPGQTFRGPDMTIFYSSQLGTYPYYTETGEPVFGGLPQNASLIAHLARTFQDILAAIPAPDFSGLAVIDWEAWRPRWAFNWDTKDIYRQRSRALVQAQHPDWPAPQVEAVAQDQFQGAARAWMAGTLQLGRALRPRGLWGFYGFPDCYNYDFLSPNYTGQCPSGIRAQNDQLGWLWGQSRALYPSIYMPAVLEGTGKSQMYVQHRVAEAFRVAVAAGDPNLPVLPYVQIFYDTTNHFLPLDELEHSLGESAAQGAAGVVLWVSWENTRTKESCQAIKEYMDTTLGPFILNVTSGALLCSQALCSGHGRCVRRTSHPKALLLLNPASFSIQLTPGGGPLSLRGALSLEDQAQMAVEFKCRCYPGWQAPWCERKSMW

SEQ ID NO: 13 - protein, 435 aa, synthetic construct
MAAHLLPICALFLTLLDMAQGFRGPLLPNRPFTTVWNANTQWCLERHGVDVDVSVFDVVANPGQTFRGPDMTIFYSDQLGTYPYYTPTGEPVFGGLPQNASLIAHLARTFQDILAAIPAPDFSGLAVIDWEEWRPRWAFNWDTKDIYRQRSRALVQAQHPDWPAPQVEAVAQDQFQGAARAWMAGTLQLGRALRPRGLWGFYGFPDCYNYDFLSPNYTGQCPSGIRAQNDQLGWLWGQSRALYPSIYMPAVLEGTGKSQMYVQHRVAEAFRVAVAAGDPNLPVLPYVQIFYDTTNHFLPLDELEHSLGESAAQGAAGVVLWVSWENTRTKESCQAIKEYMDTTLGPFILNVTSGALLCSQALCSGHGRCVRRTSHPKALLLLNPASFSIQLTPGGGPLSLRGALSLEDQAQMAVEFKCRCYPGWQAPWCERKSMW

SEQ ID NO: 14 - protein, 435 aa, synthetic construct
MAAHLLPICALFLTLLDMAQGFRGPLLPNRPFTTVWNANTQWCLERHGVDVDVSVFDVVANPGQTFRGPDMTIFYSEQLGTYPYYTPTGEPVFGGLPQNASLIAHLARTFQDILAAIPAPDFSGLAVIDWEEWRPRWAFNWDTKDIYRQRSRALVQAQHPDWPAPQVEAVAQDQFQGAARAWMAGTLQLGRALRPRGLWGFYGFPDCYNYDFLSPNYTGQCPSGIRAQNDQLGWLWGQSRALYPSIYMPAVLEGTGKSQMYVQHRVAEAFRVAVAAGDPNLPVLPYVQIFYDTTNHFLPLDELEHSLGESAAQGAAGVVLWVSWENTRTKESCQAIKEYMDTTLGPFILNVTSGALLCSQALCSGHGRCVRRTSHPKALLLLNPASFSIQLTPGGGPLSLRGALSLEDQAQMAVEFKCRCYPGWQAPWCERKSMW

SEQ ID NO: 15 - protein, 435 aa, synthetic construct
MAAHLLPICALFLTLLDMAQGFRGPLLPNRPFTTVWNANTQWCLERHGVDVDVSVFDVVANPGQTFRGPDMTIFYSDQLGTYPYYDPTGEPVFGGLPQNASLIAHLARTFQDILAAIPAPDFSGLAVIDWEAWRPRWAFNWDTKDIYRQRSRALVQAQHPDWPAPQVEAVAQDQFQGAARAWMAGTLQLGRALRPRGLWGFYGFPDCYNYDFLSPNYTGQCPSGIRAQNDQLGWLWGQSRALYPSIYMPAVLEGTGKSQMYVQHRVAEAFRVAVAAGDPNLPVLPYVQIFYDTTNHFLPLDELEHSLGESAAQGAAGVVLWVSWENTRTKESCQAIKEYMDTTLGPFILNVTSGALLCSQALCSGHGRCVRRTSHPKALLLLNPASFSIQLTPGGGPLSLRGALSLEDQAQMAVEFKCRCYPGWQAPWCERKSMW

SEQ ID NO: 16 - protein, 435 aa, synthetic construct
MAAHLLPICALFLTLLDMAQGFRGPLLPNRPFTTVWNANTQWCLERHGVDVDVSVFDVVANPGQTFRGPDMTIFYSDQLGTYPYYEPTGEPVFGGLPQNASLIAHLARTFQDILAAIPAPDFSGLAVIDWEAWRPRWAFNWDTKDIYRQRSRALVQAQHPDWPAPQVEAVAQDQFQGAARAWMAGTLQLGRALRPRGLWGFYGFPDCYNYDFLSPNYTGQCPSGIRAQNDQLGWLWGQSRALYPSIYMPAVLEGTGKSQMYVQHRVAEAFRVAVAAGDPNLPVLPYVQIFYDTTNHFLPLDELEHSLGESAAQGAAGVVLWVSWENTRTKESCQAIKEYMDTTLGPFILNVTSGALLCSQALCSGHGRCVRRTSHPKALLLLNPASFSIQLTPGGGPLSLRGALSLEDQAQMAVEFKCRCYPGWQAPWCERKSMW

SEQ ID NO: 17 - protein, 435 aa, synthetic construct
MAAHLLPICALFLTLLDMAQGFRGPLLPNRPFTTVWNANTQWCLERHGVDVDVSVFDVVANPGQTFRGPDMTIFYSDQLGTYPYYDPTGEPVFGGLPQNASLIAHLARTFQDILAAIPAPDFSGLAVIDWEEWRPRWAFNWDTKDIYRQRSRALVQAQHPDWPAPQVEAVAQDQFQGAARAWMAGTLQLGRALRPRGLWGFYGFPDCYNYDFLSPNYTGQCPSGIRAQNDQLGWLWGQSRALYPSIYMPAVLEGTGKSQMYVQHRVAEAFRVAVAAGDPNLPVLPYVQIFYDTTNHFLPLDELEHSLGESAAQGAAGVVLWVSWENTRTKESCQAIKEYMDTTLGPFILNVTSGALLCSQALCSGHGRCVRRTSHPKALLLLNPASFSIQLTPGGGPLSLRGALSLEDQAQMAVEFKCRCYPGWQAPWCERKSMW

SEQ ID NO: 18 - protein, 435 aa, synthetic construct
MAAHLLPICALFLTLLDMAQGFRGPLLPNRPFTTVWNANTQWCLERHGVDVDVSVFDVVANPGQTFRGPDMTIFYSSQLGTYPYYTPTGEPVFGGLPQNASLIAHLARTFQDILAAIPAPDFSGLAVIDWEAWRPRWARNWDTKDIYRQRSRALVQAQHPDWPAPQVEAVAQDQFQGAARAWMAGTLQLGRALRPRGLWGFYGFPDCYNYDFLSPNYTGQCPSGIRAQNDQLGWLWGQSRALYPSIYMPAVLEGTGKSQMYVQHRVAEAFRVAVAAGDPNLPVLPYVQIFYDTTNHFLPLDELEHSLGESAAQGAAGVVLWVSWENTRTKESCQAIKEYMDTTLGPFILNVTSGALLCSQALCSGHGRCVRRTSHPKALLLLNPASFSIQLTPGGGPLSLRGALSLEDQAQMAVEFKCRCYPGWQAPWCERKSMW

SEQ ID NO: 19 - protein, 435 aa, synthetic construct
MAAHLLPICALFLTLLDMAQGFRGPLLPNRPFTTVWNANTQWCLERHGVDVDVSVFDVVANPGQTFRGPDMTIFYSSQLGTYPYYTPTGEPVFGGLPQNASLIAHLARTFQDILAAIPAPDFSGLAVIDWEAWRPRWAFNWDTKDIYRQRSRALVQAQHPDWPAPQVEAVAQDQFQGAARAWMAGTLQLGRALRPRGLWGFYGFPDCYNHDFLSPNYTGQCPSGIRAQNDQLGWLWGQSRALYPSIYMPAVLEGTGKSQMYVQHRVAEAFRVAVAAGDPNLPVLPYVQIFYDTTNHFLPLDELEHSLGESAAQGAAGVVLWVSWENTRTKESCQAIKEYMDTTLGPFILNVTSGALLCSQALCSGHGRCVRRTSHPKALLLLNPASFSIQLTPGGGPLSLRGALSLEDQAQMAVEFKCRCYPGWQAPWCERKSMW

SEQ ID NO: 20 - protein, 435 aa, synthetic construct
MAAHLLPICALFLTLLDMAQGFRGPLLPNRPFTTVWNANTQWCLERHGVDVDVSVFDVVANPGQTFRGPDMTIFYSSQLGTYPYYTPTGEPVFGGLPQNASLIAHLARTFQDILAAIPAPDFSGLAVIDWEAWRPRWARNWDTKDIYRQRSRALVQAQHPDWPAPQVEAVAQDQFQGAARAWMAGTLQLGRALRPRGLWGFYGFPDCYNYDFLSPNYTGQCPSGDRAQNDQLGWLWGQSRALYPSIYMPAVLEGTGKSQMYVQHRVAEAFRVAVAAGDPNLPVLPYVQIFYDTTNHFLPLDELEHSLGESAAQGAAGVVLWVSWENTRTKESCQAIKEYMDTTLGPFILNVTSGALLCSQALCSGHGRCVRRTSHPKALLLLNPASFSIQLTPGGGPLSLRGALSLEDQAQMAVEFKCRCYPGWQAPWCERKSMW

SEQ ID NO: 21 - DNA, 32 bp, synthetic construct
  source 1..32: mol_type = other DNA
ctcgaggccaccatggcagcccacctgcttcc

SEQ ID NO: 22 - DNA, 37 bp, synthetic construct
  source 1..37: mol_type = other DNA
gcggccgctcagtggtgatggtgatgatgccacatgc

SEQ ID NO: 23 - DNA, 22 bp, synthetic construct
  source 1..22: mol_type = other DNA
caattttctatagcgaccagct

SEQ ID NO: 24 - DNA, 22 bp, synthetic construct
  source 1..22: mol_type = other DNA
agctggtcgctatagaaaattg

SEQ ID NO: 25 - DNA, 18 bp, synthetic construct
  source 1..18: mol_type = other DNA
ctatagcgagcagctggg

SEQ ID NO: 26 - DNA, 16 bp, synthetic construct
  source 1..16: mol_type = other DNA
cccagctgctcgctat

SEQ ID NO: 27 - DNA, 21 bp, synthetic construct
  source 1..21: mol_type = other DNA
ctacccctactacgatcccac

SEQ ID NO: 28 - DNA, 20 bp, synthetic construct
  source 1..20: mol_type = other DNA
ccccagtgggatcgtagtag

SEQ ID NO: 29 - DNA, 21 bp, synthetic construct
  source 1..21: mol_type = other DNA
ctacccctactacgagcccac

SEQ ID NO: 30 - DNA, 20 bp, synthetic construct
  source 1..20: mol_type = other DNA
ccccagtgggctcgtagtag

SEQ ID NO: 31 - DNA, 20 bp, synthetic construct
  source 1..20: mol_type = other DNA
ccctactacacggaaactgg

SEQ ID NO: 32 - DNA, 17 bp, synthetic construct
  source 1..17: mol_type = other DNA
gctccccagtttccgtg

SEQ ID NO: 33 - DNA, 19 bp, synthetic construct
  source 1..19: mol_type = other DNA
tgggaggaatggcgcccac

SEQ ID NO: 34 - DNA, 19 bp, synthetic construct
  source 1..19: mol_type = other DNA
gtgggcgccattcctccca

SEQ ID NO: 35 - DNA, 19 bp, synthetic construct
  source 1..19: mol_type = other DNA
tgggagaactggcgcccac

SEQ ID NO: 36 - DNA, 19 bp, synthetic construct
  source 1..19: mol_type = other DNA
gtgggcgccagttctccca

SEQ ID NO: 37 - DNA, 21 bp, synthetic construct
  source 1..21: mol_type = other DNA
catcgactgggaggattggcg

SEQ ID NO: 38 - DNA, 21 bp, synthetic construct
  source 1..21: mol_type = other DNA
cgccaatcctcccagtcgatg

SEQ ID NO: 39 - DNA, 22 bp, synthetic construct
  source 1..22: mol_type = other DNA
catcgactgggagtattggcgc

SEQ ID NO: 40 - DNA, 22 bp, synthetic construct
  source 1..22: mol_type = other DNA
gcgccaatactcccagtcgatg

SEQ ID NO: 41 - DNA, 21 bp, synthetic construct
  source 1..21: mol_type = other DNA
catcgactgggagagttggcg

SEQ ID NO: 42 - DNA, 21 bp, synthetic construct
  source 1..21: mol_type = other DNA
cgccaactctcccagtcgatg

SEQ ID NO: 43 - DNA, 21 bp, synthetic construct
  source 1..21: mol_type = other DNA
catcgactgggagcattggcg

SEQ ID NO: 44 - DNA, 21 bp, synthetic construct
  source 1..21: mol_type = other DNA
cgccaatgctcccagtcgatg

SEQ ID NO: 45 - DNA, 20 bp, synthetic construct
  source 1..20: mol_type = other DNA
cacgctgggccagaaactgg

SEQ ID NO: 46 - DNA, 21 bp, synthetic construct
  source 1..21: mol_type = other DNA
ggtgtcccagtttctggccca

SEQ ID NO: 47 - DNA, 21 bp, synthetic construct
  source 1..21: mol_type = other DNA
cctgactgctacaaccatgac

SEQ ID NO: 48 - DNA, 23 bp, synthetic construct
  source 1..23: mol_type = other DNA
gcttagaaagtcatggttgtagc

SEQ ID NO: 49 - DNA, 19 bp, synthetic construct
  source 1..19: mol_type = other DNA
gcccatcaggcgaccgtgc

SEQ ID NO: 50 - DNA, 23 bp, synthetic construct
  source 1..23: mol_type = other DNA
gtcattttgggcacggtcgcctg